European Patent Application EP 4 389 150 A1, published June 26, 2024. Title: Conjugate compounds and their use in cancer treatment and diagnosis. Applicant: Technische Universität München. The sequence listing filed with the application follows.

SEQUENCE LISTING (14 sequences)

SEQ ID NO: 1 - protein, 5 aa, synthetic construct
  REGION 1..5: note = Asp-Tyr-Phe-Phe are D-amino acids, Xaa = Ahx (aminohexanoic acid)
  SITE 5: note = misc_feature - Xaa can be any naturally occurring amino acid
DYFFX

SEQ ID NO: 2 - skipped

SEQ ID NO: 3 - protein, 6 aa, synthetic construct
  REGION 1..6: note = Lys-Asp-Tyr-Phe-Phe are D-amino acids, Xaa = Ahx (aminohexanoicacid)
  SITE 6: note = misc_feature - Xaa can be any naturally occurring amino acid
KDYFFX

SEQ ID NO: 4 - protein, 6 aa, synthetic construct
  REGION 1..6: note = Lys-Asp-Tyr-Phe are D-amino acids, Xaa-Xaa is L-Nal-Ahx(L-naphthylalanine - aminohexanoic acid)
  REGION 5..6: note = misc_feature - Xaa can be any naturally occurring amino acid
KDYFXX

SEQ ID NO: 5 - protein, 7 aa, synthetic construct
  REGION 1..7: note = Lys-Asp-Tyr-Phe-Phe are D-amino acids, Xaa-Xaa is Ahx-Ahx(aminohexanoic acid -aminohexanoic acid)
  REGION 6..7: note = misc_feature - Xaa can be any naturally occurring amino acid
KDYFFXX

SEQ ID NO: 6 - skipped

SEQ ID NO: 7 - protein, 7 aa, synthetic construct
  REGION 1..7: note = Asp-Asp-Tyr-Phe-Phe are D-amino acids, Xaa-Xaa is Ahx-Ahx(aminohexanoic acid -aminohexanoic acid)
  REGION 6..7: note = misc_feature - Xaa can be any naturally occurring amino acid
DDYFFXX

SEQ ID NO: 8 - protein, 7 aa, synthetic construct
  REGION 1..7: note = Lys-Asp-Asp are D-amino acids, Ala is beta-Ala, Xaa-Xaa isTXA-L-Nal (trans-4-(aminomethyl)-cyclohexanecarboxylic acid -L-naphthylalanine) and Lys is D-Lys
  REGION 5..6: note = misc_feature - Xaa can be any naturally occurring amino acid
KDDAXXK

SEQ ID NO: 9 - protein, 8 aa, synthetic construct
  REGION 1..8: note = Lys-Asp-Asp-Tyr-Phe-Phe are D-amino acids, Xaa is Ahx(aminohexanoic acid) and Lys is D-Lys
  SITE 7: note = misc_feature - Xaa can be any naturally occurring amino acid
KDDYFFXK

SEQ ID NO: 10 - protein, 6 aa, synthetic construct
  REGION 1..6: note = Asp-Asp are D-amino acids, Ala is beta-Ala, Xaa-Xaa is TXA-L-Nal(trans-4-(aminomethyl)-cyclohexanecarboxylic acid -L-naphthylalanine) and Lys is D-Lys
  REGION 4..5: note = misc_feature - Xaa can be any naturally occurring amino acid
DDAXXK

SEQ ID NO: 11 - protein, 7 aa, synthetic construct
  REGION 1..7: note = Xaa = D-Lys(D-Lys);Asp-Asp-Tyr-Phe-Phe are D-amino acids andXaa = Ahx (aminohexanoiic acid)
  SITE 1: note = misc_feature - Xaa can be any naturally occurring amino acid
  SITE 7: note = misc_feature - Xaa can be any naturally occurring amino acid
XDDYFFX

SEQ ID NO: 12 - protein, 7 aa, synthetic construct
  REGION 1..7: note = Xaa = D-Lys(D-Lys), Asp-Asp-Tyr-Phe are D-amino acids, Xaa-Xaa isL-Nal-Ahx (L-naphthylalanine - aminohexanoic acid)
  SITE 1: note = misc_feature - Xaa can be any naturally occurring amino acid
  REGION 6..7: note = misc_feature - Xaa can be any naturally occurring amino acid
XDDYFXX

SEQ ID NO: 13 - protein, 8 aa, synthetic construct
  REGION 1..8: note = Xaa = D-Lys(D-Lys), Asp-Asp-Tyr-Phe-Phe are D-amino acids,Xaa-Xaa is Ahx-Ahx (aminohexanoic acid - aminohexanoic acid)
  SITE 1: note = misc_feature - Xaa can be any naturally occurring amino acid
  REGION 7..8: note = misc_feature - Xaa can be any naturally occurring amino acid
XDDYFFXX

SEQ ID NO: 14 - protein, 7 aa, synthetic construct
  REGION 1..7: note = Xaa = D-Lys(D-Lys), Asp-Asp are D-amino acids, Ala is beta-Ala,Xaa-Xaa is TXA-L-Nal (trans-4-(aminomethyl)-cyclohexanecarboxylicacid - L-naphthylalanine) and Lys is D-Lys
  SITE 1: note = misc_feature - Xaa can be any naturally occurring amino acid
  REGION 5..6: note = misc_feature - Xaa can be any naturally occurring amino acid
XDDAXXK